European Patent Application EP 4 174 181 A1, published May 3, 2023. Title: SCREENING MODEL AND METHOD FOR HBV cccDNA-TARGETING DRUG. Applicant: XIAMEN UNIVERSITY YANG SHENG TANG COMPANY, LTD. Application PCT/CN2021/101986. The sequence listing filed with the application follows.

SEQUENCE LISTING (35 sequences)

SEQ ID NO: 1 - DNA, 3344 bp, Artificial sequence
  HBV 1.1-fold genome sequence
ttcacctctgcctaatcatctcttgttcatgtcctactgttcaagcctccaagctgtgccttgggtggctttggggcatggacatcgacccttataaagaatttggagctactgtggagttactctcgtttttgccttctgacttctttccttcagtacgagatcttctagataccgcctcagctctgtatcgggaagccttagagtctcctgagcattgttcacctcaccatactgcactcaggcaagcaattctttgctggggggaactaatgactctagctacctgggtgggtgttaatttggaagatccagcgtctagagacctagtagtcagttatgtcaacactaatatgggcctaaagttcaggcaactcttgtggtttcacatttcttgtctcacttttggaagagaaacagttatagagtatttggtgtctttcggagtgtggattcgcactcctccagcttatagaccaccaaatgcccctatcctatcaacacttccggagactactgttgttagacgacgaggcaggtcccctagaagaagaactccctcgcctcgcagacgaaggtctcaatcgccgcgtcgcagaagatctcaatctcgggaatctcaatgttagtattccttggactcataaggtggggaactttactgggctttattcttctactgtacctgtctttaatcctcattggaaaacaccatcttttcctaatatacatttacaccaagacattatcaaaaaatgtgaacagtttgtaggcccactcacagttaatgagaaaagaagattgcaattgattatgcctgccaggttttatccaaaggttaccaaatatttaccattggataagggtattaaaccttattatccagaacatctagttaatcattacttccaaactagacactatttacacactctatggaaggcgggtatattatataagagagaaacaacacatagcgcctcattttgtgggtcaccatattcttgggaacaagatctacagcatggggcagaatctttccaccagcaatcctctgggattctttcccgaccaccagttggatccagccttcagagcaaacaccgcaaatccagattgggacttcaatcccaacaaggacacctggccagacgccaacaaggtaggagctggagcattcgggctgggtttcaccccaccgcacggaggccttttggggtggagccctcaggctcagggcatactacaaactttgccagcaaatccgcctcctgcctccaccaatcgccagtcaggaaggcagcctaccccgctgtctccacctttgagaaacactcatcctcaggccatgcagtggaattccacaaccttccaccaaactctgcaagatcccagagtgagaggcctgtatttccctgctggtggctccagttcaggaacagtaaaccctgttctgactactgcctctcccttatcgtcaatcttctcgaggattggggaccctgcgctgaacatggagaacatcacatcaggattcctaggaccccttctcgtgttacaggcggggtttttcttgttgacaagaatcctcacaataccgcagagtctagactcgtggtggacttctctcaattttctagggggaactaccgtgtgtcttggccaaaattcgcagtccccaacctccaatcactcaccaacctcttgtcctccaacttgtcctggttatcgctggatgtgtctgcggcgttttatcatcttcctcttcatcctgctgctatgcctcatcttcttgttggttcttctggactatcaaggtatgttgcccgtttgtcctctaattccaggatcctcaacaaccagcacgggaccatgccggacctgcatgactactgctcaaggaacctctatgtatccctcctgttgctgtaccaaaccttcggacggaaattgcacctgtattcccatcccatcatcctgggctttcggaaaattcctatgggagtgggcctcagcccgtttctcctggctcagtttactagtgccatttgttcagtggttcgtagggctttcccccactgtttggctttcagttatatggatgatgtggtattgggggccaagtctgtacagcatcttgagtccctttttaccgctgttaccaattttcttttgtctttgggtatacatttaaaccctaacaaaacaaagagatggggttactctctaaattttatgggttatgtcattggatgttatgggtccttgccacaagaacacatcatacaaaaaatcaaagaatgttttagaaaacttcctattaacaggcctattgattggaaagtatgtcaacgaattgtgggtcttttgggttttgctgccccttttacacaatgtggttatcctgcgttgatgcctttgtatgcatgtattcaatctaagcaggctttcactttctcgccaacttacaaggcctttctgtgtaaacaatacctgaacctttaccccgttgcccggcaacggccaggtctgtgccaagtgtttgctgacgcaacccccactggctggggcttggtcatgggccatcagcgcatgcgtggaaccttttcggctcctctgccgatccatactgcggaactcctagccgcttgttttgctcgcagcaggtctggagcaaacattatcgggactgataactctgttgtcctatcccgcaaatatacatcgtttccatggctgctaggctgtgctgccaactggatcctgcgcgggacgtcctttgtttacgtcccgtcggcgctgaatcctgcggacgacccttctcggggtcgcttgggactctctcgtccccttctccgtctgccgttccgaccgaccacggggcgcacctctctttacgcggactccccgtctgtgccttctcatctgccggaccgtgtgcacttcgcttcacctctgcacgtcgcatggagaccaccgtgaacgcccaccaaatattgcccaaggtcttacataagaggactcttggactctcagcaatgtcaacgaccgaccttgaggcatacttcaaagactgtttgtttaaagactgggaggagttgggggaggagattaggttaaaggtctttgtactaggaggctgtaggcataaattggtctgcgcaccagcaccatgcaactttttcacctctgcctaatcatctcttgttcatgtcctactgttcaagcctccaagctgtgccttgggtggctttggggcatggacatcgacccttataaagaatttggagctactgtggagttactctcgtttttgccttctgacttctttccttcagtacgag

SEQ ID NO: 2 - protein, 11 aa, Artificial sequence
  Amino acid sequence of HiBiT
VSGWRLFKKIS

SEQ ID NO: 3 - DNA, 33 bp, Artificial sequence
  Nucleotide sequence of HiBiT
gtaagcggctggcggctattcaagaaaatctcc

SEQ ID NO: 4 - DNA, 117 bp, Artificial sequence
  Hibit16 insertion sequence
gtaagcggctggcggctattcaagaagattagcggcagcggcgtctccggttggagattattcaagaagatttcgggatccggggttagtgggtggcgcttgttcaagaagatcagc

SEQ ID NO: 5 - DNA, 624 bp, Artificial sequence
  TRE3G promoter
ggtggcggccgcaattctccaggcgatctgacggttcactaaacgagctctgcttatataggcctcccaccgtacacgccacctcgacatactcgagtttactccctatcagtgatagagaacgtatgaagagtttactccctatcagtgatagagaacgtatgcagactttactccctatcagtgatagagaacgtataaggagtttactccctatcagtgatagagaacgtatgaagagtttactccctatcagtgatagagaacgtatgcagactttactccctatcagtgatagagaacgtataaggagtttactccctatcagtgatagagaacgtatgaagagtttactccctatcagtgatagagaacgtatgcagactttactccctatcagtgatagagaacgtataaggagtttactccctatcagtgatagagaacgtatgaccagtttactccctatcagtgatagagaacgtatctacagtttactccctatcagtgatagagaacgtatatccagtttactccctatcagtgatagagaacgtataagctttaggcgtgtacggtgggcgcctataaaagcagagctcgtttagtgaaccggtcaacttt

SEQ ID NO: 6 - protein, 22 aa, Artificial sequence
  Amino acid sequence of P2A
GSGATNFSLLKQAGDVEENPGP

SEQ ID NO: 7 - DNA, 66 bp, Artificial sequence
  Nucleotide sequence of P2A
ggaagcggagctactaacttcagcctgctgaagcaggctggagacgtggaggagaaccctggacct

SEQ ID NO: 8 - DNA, 3488 bp, Artificial sequence
  HBV genome variant sequence containing Hibit16
ttcacctctgcctaatcatctcttgttcttgtcctactgttcaagcctccaagctgtgccttgggtggctttggggcaaggacatcggcagcggcgtaagcggctggcggctattcaagaagattagcggcagcggcgtctccggttggagattattcaagaagatttcgggatccggggttagtgggtggcgcttgttcaagaagatcagcggaggtaccatggacatcgacccttataaagaatttggagctactgtggagttactctcgtttttgccttctgacttctttccttcagtacgagatcttctagataccgcctcagctctgtatcgggaagccttagagtctcctgagcattgttcacctcaccatactgcactcaggcaagcaattctttgctggggggaactaatgactctagctacctgggtgggtgttaatttggaagatccagcgtctagagacctagtagtcagttatgtcaacactaatatgggcctaaagttcaggcaactcttgtggtttcacatttcttgtctcacttttggaagagaaacagttatagagtatttggtgtctttcggagtgtggattcgcactcctccagcttatagaccaccaaatgcccctatcctatcaacacttccggagactactgttgttagacgacgaggcaggtcccctagaagaagaactccctcgcctcgcagacgaaggtctcaatcgccgcgtcgcagaagatctcaatctcgggaatctcaatgttagtattccttggactcataaggtggggaactttactgggctttattcttctactgtacctgtctttaatcctcattggaaaacaccatcttttcctaatatacatttacaccaagacattatcaaaaaatgtgaacagtttgtaggcccactcacagttaatgagaaaagaagattgcaattgattatgcctgccaggttttatccaaaggttaccaaatatttaccattggataagggtattaaaccttattatccagaacatctagttaatcattacttccaaactagacactatttacacactctatggaaggcgggtatattatataagagagaaacaacacatagcgcctcattttgtgggtcaccatattcttgggaacaagatctacagcatggggcagaatctttccaccagcaatcctctgggattctttcccgaccaccagttggatccagccttcagagcaaacaccgcaaatccagattgggacttcaatcccaacaaggacacctggccagacgccaacaaggtaggagctggagcattcgggctgggtttcaccccaccgcacggaggccttttggggtggagccctcaggctcagggcatactacaaactttgccagcaaatccgcctcctgcctccaccaatcgccagtcaggaaggcagcctaccccgctgtctccacctttgagaaacactcatcctcaggccatgcagtggaattccacaaccttccaccaaactctgcaagatcccagagtgagaggcctgtatttccctgctggtggctccagttcaggaacagtaaaccctgttctgactactgcctctcccttatcgtcaatcttctcgaggattggggaccctgcgctgaacatggagaacatcacatcaggattcctaggaccccttctcgtgttacaggcggggtttttcttgttgacaagaatcctcacaataccgcagagtctagactcgtggtggacttctctcaattttctagggggaactaccgtgtgtcttggccaaaattcgcagtccccaacctccaatcactcaccaacctcttgtcctccaacttgtcctggttatcgctggatgtgtctgcggcgttttatcatcttcctcttcatcctgctgctatgcctcatcttcttgttggttcttctggactatcaaggtatgttgcccgtttgtcctctaattccaggatcctcaacaaccagcacgggaccatgccggacctgcatgactactgctcaaggaacctctatgtatccctcctgttgctgtaccaaaccttcggacggaaattgcacctgtattcccatcccatcatcctgggctttcggaaaattcctatgggagtgggcctcagcccgtttctcctggctcagtttactagtgccatttgttcagtggttcgtagggctttcccccactgtttggctttcagttatatggatgatgtggtattgggggccaagtctgtacagcatcttgagtccctttttaccgctgttaccaattttcttttgtctttgggtatacatttaaaccctaacaaaacaaagagatggggttactctctaaattttatgggttatgtcattggatgttatgggtccttgccacaagaacacatcatacaaaaaatcaaagaatgttttagaaaacttcctattaacaggcctattgattggaaagtatgtcaacgaattgtgggtcttttgggttttgctgccccttttacacaatgtggttatcctgcgttgatgcctttgtatgcatgtattcaatctaagcaggctttcactttctcgccaacttacaaggcctttctgtgtaaacaatacctgaacctttaccccgttgcccggcaacggccaggtctgtgccaagtgtttgctgacgcaacccccactggctggggcttggtcatgggccatcagcgcatgcgtggaaccttttcggctcctctgccgatccatactgcggaactcctagccgcttgttttgctcgcagcaggtctggagcaaacattatcgggactgataactctgttgtcctatcccgcaaatatacatcgtttccatggctgctaggctgtgctgccaactggatcctgcgcgggacgtcctttgtttacgtcccgtcggcgctgaatcctgcggacgacccttctcggggtcgcttgggactctctcgtccccttctccgtctgccgttccgaccgaccacggggcgcacctctctttacgcggactccccgtctgtgccttctcatctgccggaccgtgtgcacttcgcttcacctctgcacgtcgcatggagaccaccgtgaacgcccaccaaatattgcccaaggtcttacataagaggactcttggactctcagcaatgtcaacgaccgaccttgaggcatacttcaaagactgtttgtttaaagactgggaggagttgggggaggagattaggttaaaggtctttgtactaggaggctgtaggcataaattggtctgcgcaccagcaccatgcaactttttcacctctgcctaatcatctcttgttcatgtcctactgttcaagcctccaagctgtgccttgggtggctttggggcatggacatcgacccttataaagaatttggagctactgtggagttactctcgtttttgccttctgacttctttccttcagtacgag

SEQ ID NO: 9 - protein, 248 aa, Artificial sequence
  Amino acid sequence of Tet-On 3G
MSRLDKSKVINSALELLNGVGIEGLTTRKLAQKLGVEQPTLYWHVKNKRALLDALPIEMLDRHHTHSCPLEGESWQDFLRNNAKSYRCALLSHRDGAKVHLGTRPTEKQYETLENQLAFLCQQGFSLENALYALSAVGHFTLGCVLEEQEHQVAKEERETPTTDSMPPLLKQAIELFDRQGAEPAFLFGLELIICGLEKQLKCESGGPTDALDDFDLDMLPADALDDFDLDMLPADALDDFDLDMLPG

SEQ ID NO: 10 - DNA, 747 bp, Artificial sequence
  Nucleotide sequence of Tet-On 3G
atgagcagactggacaagagcaaagtcataaactctgctctggaattactcaatggagtcggtatcgaaggcctgacgacaaggaaactcgctcaaaagctgggagttgagcagcctaccctgtactggcacgtgaagaacaagcgggccctgctcgatgccctgccaatcgagatgctggacaggcatcatacccactcctgccccctggaaggcgagtcatggcaagactttctgcggaacaacgccaagtcataccgctgtgctctcctctcacatcgcgacggggctaaagtgcatctcggcacccgcccaacagagaaacagtacgaaaccctggaaaatcagctcgcgttcctgtgtcagcaaggcttctccctggagaacgcactgtacgctctgtccgccgtgggccactttacactgggctgcgtattggaggaacaggagcatcaagtagcaaaagaggaaagagagacacctaccaccgattctatgcccccacttctgaaacaagcaattgagctgttcgaccggcagggagccgaacctgccttccttttcggcctggaactaatcatatgtggcctggagaaacagctaaagtgcgaaagcggcgggccgaccgacgcccttgacgattttgacttagacatgctcccagccgatgcccttgacgactttgaccttgatatgctgcctgctgacgctcttgacgattttgaccttgacatgctccccgggtag

SEQ ID NO: 11 - protein, 311 aa, Artificial sequence
  Amino acid sequence of iRFP
MARKVDLTSCDREPIHIPGSIQPCGCLLACDAQAVRITRITENAGAFFGRETPRVGELLADYFGETEAHALRNALAQSSDPKRPALIFGWRDGLTGRTFDISLHRHDGTSIIEFEPAAAEQADNPLRLTRQIIARTKELKSLEEMAARVPRYLQAMLGYHRVMLYRFADDGSGMVIGEAKRSDLESFLGQHFPASLVPQQARLLYLKNAIRVVSDSRGISSRIVPEHDASGAALDLSFAHLRSISPCHLEFLRNMGVSASMSLSIIIDGTLWGLIICHHYEPRAVPMAQRVAAEMFADFLSLHFTAAHHQR

SEQ ID NO: 12 - DNA, 936 bp, Artificial sequence
  Nucleotide sequence of iRFP
atggcgcgtaaggtcgatctcacctcctgcgatcgcgagccgatccacatccccggcagcattcagccgtgcggctgcctgctggcctgcgacgcgcaggcggtgcggatcacgcgcattacggaaaatgccggcgcgttctttggacgcgaaactccgcgggtcggtgagctactcgccgattacttcggcgagaccgaagcccatgcgctgcgcaacgcactggcgcagtcctccgatccaaagcgaccggcgctgatcttcggttggcgcgacggcctgaccggccgcaccttcgacatctcactgcatcgccatgacggcaccagcatcatcgagttcgagcctgcggcggccgaacaggccgacaatccgctgcggctgacgcggcagatcatcgcgcgcaccaaagaactgaagtcgctcgaagagatggccgcacgggtgccgcgctatctgcaggcgatgctcggctatcaccgcgtgatgttgtaccgcttcgcggacgacggctccgggatggtgatcggcgaggcgaagcgcagcgacctggagagctttctcggtcagcactttccggcgtcgctggtcccgcagcaggcgcggctactgtacttgaagaacgcgatccgcgtggtctcggattcgcgcggcatcagcagccggatcgtgcccgagcacgacgcctccggcgccgcgctcgatctgtcgttcgcgcacctgcgcagcatctcgccctgccatctcgaatttctgcggaacatgggcgtcagcgcctcgatgtcgctgtcgatcatcattgacggcacgctatggggattgatcatctgtcatcattacgagccgcgtgccgtgccgatggcgcagcgcgtcgcggccgaaatgttcgccgacttcttatcgctgcacttcaccgccgcccaccaccaacgctga

SEQ ID NO: 13 - DNA, 405 bp, Artificial sequence
  Blasticidin-resistant gene
atggccaagcctttgtctcaagaagaatccaccctcattgaaagagcaacggctacaatcaacagcatccccatctctgaagactacagcgtcgccagcgcagctctctctagcgacggccgcatcttcactggtgtcaatgtatatcattttactgggggaccttgtgcagaactcgtggtgctgggcactgctgctgctgcggcagctggcaacctgacttgtatcgtcgcgatcggaaatgagaacaggggcatcttgagcccctgcggacggtgccgacaggtgcttctcgatctgcatcctgggatcaaagccatagtgaaggacagtgatggacagccgacggcagttgggattcgtgaattgctgccctctggttatgtgtgggagggctgagcttga

SEQ ID NO: 14 - DNA, 306 bp, Artificial sequence
  Rccc1a  Sequence of 3' end region of C-ORF of HBV genome
gacctagtagtcagttatgtcaacactaatatgggcctaaagttcaggcaactcttgtggtttcacatttcttgtctcacttttggaagagaaacagttatagagtatttggtgtctttcggagtgtggattcgcactcctccagcttatagaccaccaaatgcccctatcctatcaacacttccggagactactgttgttagacgacgaggcaggtcccctagaagaagaactccctcgcctcgcagacgaaggtctcaatcgccgcgtcgcagaagatctcaatctcgggaatctcaatgttag

SEQ ID NO: 15 - DNA, 147 bp, Artificial sequence
  Rccc1a  Sequence of 5' end region of C-ORF of HBV genome
cttctagataccgcctcagctctgtatcgggaagccttagagtctcctgagcattgttcacctcaccatactgcactcaggcaagcaattctttgctggggggaactaatgactctagctacctgggtgggtgttaatttggaagat

SEQ ID NO: 16 - DNA, 2717 bp, Artificial sequence
  Rccc1a  Sequence of HBV genome fragment in which C-ORF is removed
tattccttggactcataaggtggggaactttactgggctttattcttctactgtacctgtctttaatcctcattggaaaacaccatcttttcctaatatacatttacaccaagacattatcaaaaaatgtgaacagtttgtaggcccactcacagttaatgagaaaagaagattgcaattgattatgcctgccaggttttatccaaaggttaccaaatatttaccattggataagggtattaaaccttattatccagaacatctagttaatcattacttccaaactagacactatttacacactctatggaaggcgggtatattatataagagagaaacaacacatagcgcctcattttgtgggtcaccatattcttgggaacaagatctacagcatggggcagaatctttccaccagcaatcctctgggattctttcccgaccaccagttggatccagccttcagagcaaacaccgcaaatccagattgggacttcaatcccaacaaggacacctggccagacgccaacaaggtaggagctggagcattcgggctgggtttcaccccaccgcacggaggccttttggggtggagccctcaggctcagggcatactacaaactttgccagcaaatccgcctcctgcctccaccaatcgccagtcaggaaggcagcctaccccgctgtctccacctttgagaaacactcatcctcaggccatgcagtggaattccacaaccttccaccaaactctgcaagatcccagagtgagaggcctgtatttccctgctggtggctccagttcaggaacagtaaaccctgttctgactactgcctctcccttatcgtcaatcttctcgaggattggggaccctgcgctgaacatggagaacatcacatcaggattcctaggaccccttctcgtgttacaggcggggtttttcttgttgacaagaatcctcacaataccgcagagtctagactcgtggtggacttctctcaattttctagggggaactaccgtgtgtcttggccaaaattcgcagtccccaacctccaatcactcaccaacctcttgtcctccaacttgtcctggttatcgctggatgtgtctgcggcgttttatcatcttcctcttcatcctgctgctatgcctcatcttcttgttggttcttctggactatcaaggtatgttgcccgtttgtcctctaattccaggatcctcaacaaccagcacgggaccatgccggacctgcatgactactgctcaaggaacctctatgtatccctcctgttgctgtaccaaaccttcggacggaaattgcacctgtattcccatcccatcatcctgggctttcggaaaattcctatgggagtgggcctcagcccgtttctcctggctcagtttactagtgccatttgttcagtggttcgtagggctttcccccactgtttggctttcagttatatggatgatgtggtattgggggccaagtctgtacagcatcttgagtccctttttaccgctgttaccaattttcttttgtctttgggtatacatttaaaccctaacaaaacaaagagatggggttactctctaaattttatgggttatgtcattggatgttatgggtccttgccacaagaacacatcatacaaaaaatcaaagaatgttttagaaaacttcctattaacaggcctattgattggaaagtatgtcaacgaattgtgggtcttttgggttttgctgccccttttacacaatgtggttatcctgcgttgatgcctttgtatgcatgtattcaatctaagcaggctttcactttctcgccaacttacaaggcctttctgtgtaaacaatacctgaacctttaccccgttgcccggcaacggccaggtctgtgccaagtgtttgctgacgcaacccccactggctggggcttggtcatgggccatcagcgcatgcgtggaaccttttcggctcctctgccgatccatactgcggaactcctagccgcttgttttgctcgcagcaggtctggagcaaacattatcgggactgataactctgttgtcctatcccgcaaatatacatcgtttccatggctgctaggctgtgctgccaactggatcctgcgcgggacgtcctttgtttacgtcccgtcggcgctgaatcctgcggacgacccttctcggggtcgcttgggactctctcgtccccttctccgtctgccgttccgaccgaccacggggcgcacctctctttacgcggactccccgtctgtgccttctcatctgccggaccgtgtgcacttcgcttcacctctgcacgtcgcatggagaccaccgtgaacgcccaccaaatattgcccaaggtcttacataagaggactcttggactctcagcaatgtcaacgaccgaccttgaggcatacttcaaagactgtttgtttaaagactgggaggagttgggggaggagattaggttaaaggtctttgtactaggaggctgtaggcataaattggtctgcgcaccagcaccatgcaactttttcacctctgcctaatcatctcttgttcatgtcctactgttcaagcctccaagctgtgccttgggtggctttggggcatggacatcgacccttataaagaatttggagctactgtggagttactctcgtttttgccttctgacttctttccttcagtacgagat

SEQ ID NO: 17 - DNA, 3324 bp, Artificial sequence
  Rccc1a linear replicon sequence
ataacttcgtataatgtatgctatacgaagttatctggcggtagcggtgtgagcggctggcgcctgttcaagaagatcagcggcggcggcggcagcaccggtgacctagtagtcagttatgtcaacactaatatgggcctaaagttcaggcaactcttgtggtttcacatttcttgtctcacttttggaagagaaacagttatagagtatttggtgtctttcggagtgtggattcgcactcctccagcttatagaccaccaaatgcccctatcctatcaacacttccggagactactgttgttagacgacgaggcaggtcccctagaagaagaactccctcgcctcgcagacgaaggtctcaatcgccgcgtcgcagaagatctcaatctcgggaatctcaatgttagtattccttggactcataaggtggggaactttactgggctttattcttctactgtacctgtctttaatcctcattggaaaacaccatcttttcctaatatacatttacaccaagacattatcaaaaaatgtgaacagtttgtaggcccactcacagttaatgagaaaagaagattgcaattgattatgcctgccaggttttatccaaaggttaccaaatatttaccattggataagggtattaaaccttattatccagaacatctagttaatcattacttccaaactagacactatttacacactctatggaaggcgggtatattatataagagagaaacaacacatagcgcctcattttgtgggtcaccatattcttgggaacaagatctacagcatggggcagaatctttccaccagcaatcctctgggattctttcccgaccaccagttggatccagccttcagagcaaacaccgcaaatccagattgggacttcaatcccaacaaggacacctggccagacgccaacaaggtaggagctggagcattcgggctgggtttcaccccaccgcacggaggccttttggggtggagccctcaggctcagggcatactacaaactttgccagcaaatccgcctcctgcctccaccaatcgccagtcaggaaggcagcctaccccgctgtctccacctttgagaaacactcatcctcaggccatgcagtggaattccacaaccttccaccaaactctgcaagatcccagagtgagaggcctgtatttccctgctggtggctccagttcaggaacagtaaaccctgttctgactactgcctctcccttatcgtcaatcttctcgaggattggggaccctgcgctgaacatggagaacatcacatcaggattcctaggaccccttctcgtgttacaggcggggtttttcttgttgacaagaatcctcacaataccgcagagtctagactcgtggtggacttctctcaattttctagggggaactaccgtgtgtcttggccaaaattcgcagtccccaacctccaatcactcaccaacctcttgtcctccaacttgtcctggttatcgctggatgtgtctgcggcgttttatcatcttcctcttcatcctgctgctatgcctcatcttcttgttggttcttctggactatcaaggtatgttgcccgtttgtcctctaattccaggatcctcaacaaccagcacgggaccatgccggacctgcatgactactgctcaaggaacctctatgtatccctcctgttgctgtaccaaaccttcggacggaaattgcacctgtattcccatcccatcatcctgggctttcggaaaattcctatgggagtgggcctcagcccgtttctcctggctcagtttactagtgccatttgttcagtggttcgtagggctttcccccactgtttggctttcagttatatggatgatgtggtattgggggccaagtctgtacagcatcttgagtccctttttaccgctgttaccaattttcttttgtctttgggtatacatttaaaccctaacaaaacaaagagatggggttactctctaaattttatgggttatgtcattggatgttatgggtccttgccacaagaacacatcatacaaaaaatcaaagaatgttttagaaaacttcctattaacaggcctattgattggaaagtatgtcaacgaattgtgggtcttttgggttttgctgccccttttacacaatgtggttatcctgcgttgatgcctttgtatgcatgtattcaatctaagcaggctttcactttctcgccaacttacaaggcctttctgtgtaaacaatacctgaacctttaccccgttgcccggcaacggccaggtctgtgccaagtgtttgctgacgcaacccccactggctggggcttggtcatgggccatcagcgcatgcgtggaaccttttcggctcctctgccgatccatactgcggaactcctagccgcttgttttgctcgcagcaggtctggagcaaacattatcgggactgataactctgttgtcctatcccgcaaatatacatcgtttccatggctgctaggctgtgctgccaactggatcctgcgcgggacgtcctttgtttacgtcccgtcggcgctgaatcctgcggacgacccttctcggggtcgcttgggactctctcgtccccttctccgtctgccgttccgaccgaccacggggcgcacctctctttacgcggactccccgtctgtgccttctcatctgccggaccgtgtgcacttcgcttcacctctgcacgtcgcatggagaccaccgtgaacgcccaccaaatattgcccaaggtcttacataagaggactcttggactctcagcaatgtcaacgaccgaccttgaggcatacttcaaagactgtttgtttaaagactgggaggagttgggggaggagattaggttaaaggtctttgtactaggaggctgtaggcataaattggtctgcgcaccagcaccatgcaactttttcacctctgcctaatcatctcttgttcatgtcctactgttcaagcctccaagctgtgccttgggtggctttggggcatggacatcgacccttataaagaatttggagctactgtggagttactctcgtttttgccttctgacttctttccttcagtacgagatcttctagataccgcctcagctctgtatcgggaagccttagagtctcctgagcattgttcacctcaccatactgcactcaggcaagcaattctttgctggggggaactaatgactctagctacctgggtgggtgttaatttggaagatggaggtaccggcggtagcataacttcgtataatgtatgctatacgaagttat

SEQ ID NO: 18 - DNA, 3290 bp, Artificial sequence
  Rccc1a recombinant cccDNA sequence
ataacttcgtataatgtatgctatacgaagttatctggcggtagcggtgtgagcggctggcgcctgttcaagaagatcagcggcggcggcggcagcaccggtgacctagtagtcagttatgtcaacactaatatgggcctaaagttcaggcaactcttgtggtttcacatttcttgtctcacttttggaagagaaacagttatagagtatttggtgtctttcggagtgtggattcgcactcctccagcttatagaccaccaaatgcccctatcctatcaacacttccggagactactgttgttagacgacgaggcaggtcccctagaagaagaactccctcgcctcgcagacgaaggtctcaatcgccgcgtcgcagaagatctcaatctcgggaatctcaatgttagtattccttggactcataaggtggggaactttactgggctttattcttctactgtacctgtctttaatcctcattggaaaacaccatcttttcctaatatacatttacaccaagacattatcaaaaaatgtgaacagtttgtaggcccactcacagttaatgagaaaagaagattgcaattgattatgcctgccaggttttatccaaaggttaccaaatatttaccattggataagggtattaaaccttattatccagaacatctagttaatcattacttccaaactagacactatttacacactctatggaaggcgggtatattatataagagagaaacaacacatagcgcctcattttgtgggtcaccatattcttgggaacaagatctacagcatggggcagaatctttccaccagcaatcctctgggattctttcccgaccaccagttggatccagccttcagagcaaacaccgcaaatccagattgggacttcaatcccaacaaggacacctggccagacgccaacaaggtaggagctggagcattcgggctgggtttcaccccaccgcacggaggccttttggggtggagccctcaggctcagggcatactacaaactttgccagcaaatccgcctcctgcctccaccaatcgccagtcaggaaggcagcctaccccgctgtctccacctttgagaaacactcatcctcaggccatgcagtggaattccacaaccttccaccaaactctgcaagatcccagagtgagaggcctgtatttccctgctggtggctccagttcaggaacagtaaaccctgttctgactactgcctctcccttatcgtcaatcttctcgaggattggggaccctgcgctgaacatggagaacatcacatcaggattcctaggaccccttctcgtgttacaggcggggtttttcttgttgacaagaatcctcacaataccgcagagtctagactcgtggtggacttctctcaattttctagggggaactaccgtgtgtcttggccaaaattcgcagtccccaacctccaatcactcaccaacctcttgtcctccaacttgtcctggttatcgctggatgtgtctgcggcgttttatcatcttcctcttcatcctgctgctatgcctcatcttcttgttggttcttctggactatcaaggtatgttgcccgtttgtcctctaattccaggatcctcaacaaccagcacgggaccatgccggacctgcatgactactgctcaaggaacctctatgtatccctcctgttgctgtaccaaaccttcggacggaaattgcacctgtattcccatcccatcatcctgggctttcggaaaattcctatgggagtgggcctcagcccgtttctcctggctcagtttactagtgccatttgttcagtggttcgtagggctttcccccactgtttggctttcagttatatggatgatgtggtattgggggccaagtctgtacagcatcttgagtccctttttaccgctgttaccaattttcttttgtctttgggtatacatttaaaccctaacaaaacaaagagatggggttactctctaaattttatgggttatgtcattggatgttatgggtccttgccacaagaacacatcatacaaaaaatcaaagaatgttttagaaaacttcctattaacaggcctattgattggaaagtatgtcaacgaattgtgggtcttttgggttttgctgccccttttacacaatgtggttatcctgcgttgatgcctttgtatgcatgtattcaatctaagcaggctttcactttctcgccaacttacaaggcctttctgtgtaaacaatacctgaacctttaccccgttgcccggcaacggccaggtctgtgccaagtgtttgctgacgcaacccccactggctggggcttggtcatgggccatcagcgcatgcgtggaaccttttcggctcctctgccgatccatactgcggaactcctagccgcttgttttgctcgcagcaggtctggagcaaacattatcgggactgataactctgttgtcctatcccgcaaatatacatcgtttccatggctgctaggctgtgctgccaactggatcctgcgcgggacgtcctttgtttacgtcccgtcggcgctgaatcctgcggacgacccttctcggggtcgcttgggactctctcgtccccttctccgtctgccgttccgaccgaccacggggcgcacctctctttacgcggactccccgtctgtgccttctcatctgccggaccgtgtgcacttcgcttcacctctgcacgtcgcatggagaccaccgtgaacgcccaccaaatattgcccaaggtcttacataagaggactcttggactctcagcaatgtcaacgaccgaccttgaggcatacttcaaagactgtttgtttaaagactgggaggagttgggggaggagattaggttaaaggtctttgtactaggaggctgtaggcataaattggtctgcgcaccagcaccatgcaactttttcacctctgcctaatcatctcttgttcatgtcctactgttcaagcctccaagctgtgccttgggtggctttggggcatggacatcgacccttataaagaatttggagctactgtggagttactctcgtttttgccttctgacttctttccttcagtacgagatcttctagataccgcctcagctctgtatcgggaagccttagagtctcctgagcattgttcacctcaccatactgcactcaggcaagcaattctttgctggggggaactaatgactctagctacctgggtgggtgttaatttggaagatggaggtaccggcggtagc

SEQ ID NO: 19 - DNA, 34 bp, Artificial sequence
  loxP sequence
ataacttcgtatagcatacattatacgaagttat

SEQ ID NO: 20 - protein, 380 aa, Artificial sequence
  Amino acid sequence of Cre recombinase
MGHHHHHHGMGAAGRKKRRQRRRPPAGTSVSLKKKRKVSNLLTVHQNLPALPVDATSDEVRKNLMDMFRDRQAFSEHTWKMLLSVCRSWAAWCKLNNRKWFPAEPEDVRDYLLYLQARGLAVKTIQQHLGQLNMLHRRSGLPRPSDSNAVSLVMRRIRKENVDAGERAKQALAFERTDFDQVRSLMENSDRCQDIRNLAFLGIAYNTLLRIAEIARIRVKDISRTDGGRMLIHIGRTKTLVSTAGVEKALSLGVTKLVERWISVSGVADDPNNYLFCRVRKNGVAAPSATSQLSTRALEGIFEATHRLIYGAKDDSGQRYLAWSGHSARVGAARDMARAGVSIPEIMQAGGWTNVNIVMNYIRNLDSETGAMVRLLEDGD

SEQ ID NO: 21 - DNA, 1143 bp, Artificial sequence
  Nucleotide sequence of Cre recombinase
atgggccatcaccatcaccatcacggcatgggcgctgcaggtcgcaagaaacgtcgccaacgtcgccgtccgcctgcaggcactagtgtaagcttgaagaagaagaggaaggtgtccaatttactgaccgtacaccaaaatttgcctgcattaccggtcgatgcaacgagtgatgaggttcgcaagaacctgatggacatgttcagggatcgccaggcgttttctgagcatacctggaaaatgcttctgtccgtttgccggtcgtgggcggcatggtgcaagttgaataaccggaaatggtttcccgcagaacctgaagatgttcgcgattatcttctatatcttcaggcgcgcggtctggcagtaaaaactatccagcaacatttgggccagctaaacatgcttcatcgtcggtccgggctgccacgaccaagtgacagcaatgctgtttcactggttatgcggcggatccgaaaagaaaacgttgatgccggtgaacgtgcaaaacaggctctagcgttcgaacgcactgatttcgaccaggttcgttcactcatggaaaatagcgatcgctgccaggatatacgtaatctggcatttctggggattgcttataacaccctgttacgtatagccgaaattgccaggatcagggttaaagatatctcacgtactgacggtgggagaatgttaatccatattggcagaacgaaaacgctggttagcaccgcaggtgtagagaaggcacttagcctgggggtaactaaactggtcgagcgatggatttccgtctctggtgtagctgatgatccgaataactacctgttttgccgggtcagaaaaaatggtgttgccgcgccatctgccaccagccagctatcaactcgcgccctggaagggatttttgaagcaactcatcgattgatttacggcgctaaggatgactctggtcagagatacctggcctggtctggacacagtgcccgtgtcggagccgcgcgagatatggcccgcgctggagtttcaataccggagatcatgcaagctggtggctggaccaatgtaaatattgtcatgaactatatccgtaacctggatagtgaaacaggggcaatggtgcgcctgctggaagatggcgattag

SEQ ID NO: 22 - DNA, 20 bp, Artificial sequence
  HBV-F
tttcacctctgcctaatcat

SEQ ID NO: 23 - DNA, 26 bp, Artificial sequence
  HBV-R
tcagaaggcaaaaaagagagtaactc

SEQ ID NO: 24 - DNA, 24 bp, Artificial sequence
  HBV-Probe
ccttgggtggctttggggcatgga

SEQ ID NO: 25 - DNA, 25 bp, Artificial sequence
  cccDNA-Probe
accgtgaacgcccaccgaatgttgc

SEQ ID NO: 26 - DNA, 17 bp, Artificial sequence
  cccDNA-F
tgcacttcgcttcacct

SEQ ID NO: 27 - DNA, 17 bp, Artificial sequence
  cccDNA-R
aggggcatttggtggtc

SEQ ID NO: 28 - DNA, 16 bp, Artificial sequence
  mt4987F
cccagctacgcaaaat

SEQ ID NO: 29 - DNA, 21 bp, Artificial sequence
  mt5106R
aatgcggtagtagttaggata

SEQ ID NO: 30 - DNA, 24 bp, Artificial sequence
  mt5010-Probe
catactcctcaattacccacatag

SEQ ID NO: 31 - DNA, 113 bp, Artificial Sequence
  Artificial sequence in Figure 2
tgcaactttttcacctctgcctaatcatctcttgttcttgtcctactgttcaagcctccaagctgtgccttgggtggctttggggcaaggacatcgacccttataaagaattt

SEQ ID NO: 32 - DNA, 105 bp, Artificial sequence
  Artificial sequence in Figure 2
atgcaactttttcacctctgcctaatcatctcttgttcatgtcctactgttcaagcctccaagctgtgccttgggtggctttggggcatggacatcattgacccg

SEQ ID NO: 33 - DNA, 13 bp, Artificial sequence
  Artificial sequence in Figure 2
agtggagacggat

SEQ ID NO: 34 - DNA, 20 bp, Artificial sequence
  Artificial sequence in Figure 2
tacgttgaaaaagtggagac

SEQ ID NO: 35 - DNA, 134 bp, Artificial sequence
  Artificial sequence in Figure 5
ctctagctacctgggtgggtgttaatttggaagatggaggtaccggcggtagcataacttcgtataatgtatgctatacgaagttatctggcggtagcggtgtgagcggctggcgcctgttcaagaagatcagc